European Patent Specification EP 3 298 134 B1, published May 10, 2023. Title: GENE EDITING OF DEEP INTRONIC MUTATIONS. Applicant: RUAN, Guoxiang SCARIA, Abraham. Application Not Yet Assigned. The sequence listing filed with the application follows.

SEQUENCE LISTING (66 sequences)

SEQ ID NO: 1 - DNA, 25 bp, Artificial Sequence
  Synthetic construct
caccgaagacactgccaatagggat

SEQ ID NO: 2 - DNA, 25 bp, Artificial Sequence
  Synthetic construct
aaacatccctattggcagtgtcttc

SEQ ID NO: 3 - DNA, 158 bp, Artificial Sequence
  Synthetic construct
ccacccgcctcggcctcctaaagtgctgggattacagatgtgagccaccgcacctggccccagttgtaattgtgagtatctcatacgtatccctattggcagtgtcttagttttattttttattatctttattgtggcagccattattcctgtctcta

SEQ ID NO: 4 - DNA, 20 bp, Artificial Sequence
  Synthetic construct
ggtccctggcttttgttcct

SEQ ID NO: 5 - DNA, 20 bp, Artificial Sequence
  Synthetic construct
caggaggctgagggtgtttt

SEQ ID NO: 6 - DNA, 20 bp, Artificial Sequence
  Synthetic construct
agtagagatggggtttcacc

SEQ ID NO: 7 - DNA, 26 bp, Artificial Sequence
  Synthetic construct
tgactgctaagtacagggacatcttg

SEQ ID NO: 8 - DNA, 24 bp, Artificial Sequence
  Synthetic construct
aggagatgttttcacactccaggt

SEQ ID NO: 9 - DNA, 23 bp, Artificial Sequence
  Synthetic construct
ctggccccagttgtaatttgtga

SEQ ID NO: 10 - DNA, 24 bp, Artificial Sequence
  Synthetic construct
ctgttcccaggcttgttcaatagt

SEQ ID NO: 11 - DNA, 24 bp, Artificial Sequence
  Synthetic construct
caccggcgggtggatcacgagttc

SEQ ID NO: 12 - DNA, 24 bp, Artificial Sequence
  Synthetic construct
aaacgaactcgtgatccacccgcc

SEQ ID NO: 13 - DNA, 25 bp, Artificial Sequence
  Synthetic construct
caccgaaagctaccggttacctgaa

SEQ ID NO: 14 - DNA, 25 bp, Artificial Sequence
  Synthetic construct
aaacttcaggtaaccggtagctttc

SEQ ID NO: 15 - DNA, 25 bp, Artificial Sequence
  Synthetic construct
caccgtcattcttgtggcagtaagg

SEQ ID NO: 16 - DNA, 25 bp, Artificial Sequence
  Synthetic construct
aaacccttactgccacaagaatgac

SEQ ID NO: 17 - DNA, 24 bp, Artificial Sequence
  Synthetic construct
caccggagtcacatgggagtcaca

SEQ ID NO: 18 - DNA, 24 bp, Artificial Sequence
  Synthetic construct
aaactgtgactcccatgtgactcc

SEQ ID NO: 19 - DNA, 102 bp, Artificial Sequence
  Synthetic construct
ggcgggtggatcacgagttcgttttagagctagaaatagcaagttaaaataaggctagtccgttatcaacttgaaaaagtggcaccgagtcggtgctttttt

SEQ ID NO: 20 - DNA, 103 bp, Artificial Sequence
  Synthetic construct
gaaagctaccggttacctgaagttttagagctagaaatagcaagttaaaataaggctagtccgttatcaacttgaaaaagtggcaccgagtcggtgctttttt

SEQ ID NO: 21 - DNA, 103 bp, Artificial Sequence
  Synthetic construct
gtcattcttgtggcagtaagggttttagagctagaaatagcaagttaaaataaggctagtccgttatcaacttgaaaaagtggcaccgagtcggtgctttttt

SEQ ID NO: 22 - DNA, 102 bp, Artificial Sequence
  Synthetic construct
ggagtcacatgggagtcacagttttagagctagaaatagcaagttaaaataaggctagtccgttatcaacttgaaaaagtggcaccgagtcggtgctttttt

SEQ ID NO: 23 - DNA, 5838 bp, Homo Sapiens
gtaagtttgtgtgattcttgaaccttgtgaaattagccatttttcttcaatatttttgtgtttggggggatttggcagattttaattaaagtttgcctgcatttatataaatttaacagagatataattatccatattattcattcagtttagttataaatattttgttcccacataacacacacacacacacacaatatattatctatttatagtggctgaatgacttctgaatgattatctagatcattctccttaggtcacttgcatgatttagctgaatcaaacctcttttaaccagacatctaagagaaaaaggagcatgaaacaggtagaatattgtaatcaaaggagggaagcactcattaagtgcccatccctttctcttacccctgtacccagaacaaactattctcccatggtccctggcttttgttccttggaatggatgtagccaacagtagctgaaatattaagggctcttcctggaccatggatgcactctgtaaattctcatcattttttattgtagaataaatgtagaattttaatgtagaataaatttatttaatgtagaataaaaaataaaaaaactagagtagaatatcataagttacaatctgtgaatatggaccagaccctttgtagttatcttacagccacttgaactctataccttttactgaggacagaacaagctcctgatttgttcatcttcctcatcagaaatagaggcttatggattttggattattcttatctaagatcctttcacaggagtagaataagatctaattctattagctcaaaagcttttgctggctcatagagacacattcagtaaatgaaaacgttgttctgagtagctttcaggattcctactaaattatgagtcatgtttatcaatattatttagaagtaatcataatcagtttgctttctgctgcttttgccaaagagaggtgattatgttactttttatagaaaattatgcctatttagtgtggtgataatttatttttttccattctccatgtcctctgtcctatcctctccagcattagaaagtcctaggcaagagacatcttgtggataatgtatcaatgagtgatgtttaacgttatcattttcccaaagagtatttttcatctttcctaaagattttttttttttttttttgagatggagtttcattctgtcacccaggctgagtgcagtggcacgatctcggcttaacgcttactgcatcctctgcctcccagattcaagcagttctcctgcctcagcctctgagtagctgggattacaggtgtgcaccaccacaccagctaatttttttttttttttttttttttttgaggcagagtctcgctctgtcacccaggctggagtgcagtggcgccatcttggctcactgcaagctccacctcccgggttcaggccgttctcctgcctcagcctcctgagtagctggtaccacaggcacccaccatcatgcccggctaattttttgtatttttagtagagatggggtttcaccttgttagccaggatggtgtcgatctcctgaactcgtgatccacccgcctcggcctcctaaagtgctgggattacagatgtgagccaccgcacctggccccagttgtaattgtgagtatctcatacctatccctattggcagtgtcttagttttattttttattatctttattgtggcagccattattcctgtctctatctccagtcttacatcctccttactgccacaagaatgatcattctaaacatgaatcctaccctgtgactcccatgtgactccccgccttaaaaactgtcaaaagctaccggttacctgaagggtaaaagtcaagtcccctacttacctcatgtcatctagagcaagagatgaactagctgagttttctgaccacagtgttctttcttatgtatgttcttttgtacgtgctcttttctatatatagggaaccatttctctcttccagttgttttgctcagtgaatttctattcctgtttcaaaacttgttcaggcattaccttttttttcttaagcatactttttttaatggaacaaagtcactcctgtctacactagttctgcatcttatacataggttttgtacatagtacatatttatatcacatcaaattatatgtgtttacatatctgtcttccttaatggaatataagtcttttgatataaggaactatttaatttgtttctgtgtgttgagtatctcctgtttggcacagagttcaagctaatacatgagagtgattagtggtggagagccacagtgcatgtggtgtcaaatatggtgcttaggaaattattgttgctttttgagaggtaaaggttcatgagactagaggtcacgaaaatcagatttcatgtgtgaagaatggaatagataataaggaaatacaaaaactggatgggtaataaagcaaaagaaaaacttgaaatttgatagtagaagaaaaaagaaatagatgtagattgaggtagaatcaagaagaggattctttttttgttgtttttttttttgaaacagagtctcactgtgttgcccaggctggagtgcagtggagtgatcttggcttactgcaacctctgcctcccaggttcaagcgattcttctgcttcagtctcccgagtagctggaattacaggtgcccaccagcacggccggctaatttagtagagacagggttttgccatgttggccgggctggtctcaaactttggatctcaggtaatccgccagcctcaacttcccaaagtgctgggattacaggcatgagccactgtgcccagcctgtttttttttttttaaaggagaccagtgaagtttcaggaggagggaaagaaaatttagagttactagggagagagtgatgaagataagagatgaaagtggtaataagggaaatagcaaaatatcagggtaggtgggagaaaaagagatttgtaacaaacaataggattatcctgtgaaaaaggatgaaaggaagaaaaaaatggatagaaagatatttaaaacaccctcagcctcctgttttccctcctgtgtattcatagtatataaaactataattatgtactttacttaaaaaatatattattattaccttatcgtgcttatttaatcatagcatgtcctctttttagtctcattaccctgtttgtattattcttcataacacttaatacctgacattgtattatatattggcttattttccaggtactccactcaaatataagttctaggatataatttatttatcactgaaatccattgcttagagtacctggcatgtagtaaataggcattctgttttttcaaataaaaaataaaggaacttaagatatatatttatgttatatcgccagcctttttcctcacagctctattctgttgtacagaattacctactttacaattcctgtgtttcaaggggatctcaaatttaacgtgtccacaatgaactcctgatttctgtttctctcctagtcattcttatttcaatatatgttcagttacctaaccagctagtcaaggcagatactttagagttattctgtagtcattctttttccctaccatttttgttttccaaatgtaatttatgtgtgtcttcttcatcctcgcagctctaacccttgtccaaaccagcatcatcactcatctggagttccacaatgtctttctggctagtttccctgatttctctattgacccctttattctccacagtgcagccagaatgattgtttaaaacttcctccttaaaatctttaaattgttttcttttatacgttaagttaaattccagttccttgtcttggcatgccatgccctgcctggtgtggcccctgatggtctctccaacttcatgttttactactattgactcttatttttgcttactctgcttgggtgctccagtcctccaaatcatttcctgctccaatcatttcaatcattttttcctctcagatcttatagtattccaaatgctttcttcctttggagcatctgggtttactaataaatacttcgtacctcacagttcagcttaaatatcaattatttggtggttaagacatccttcaaccgctctatctaaatgttcctttctattattcactggctcagtactctgtttttattttctttctaaatgtcaacttttttttttttgagtcagggtctcactgttgcccaggctcgagtgcagttgcacaatcatagctcattgcagccttgccctcctgggatcaagtaattctcccacctcagcctccaaaatagctgggattacaggtatgcatcaccatgctcagctaattttttgtgtttttttgtagagatgaggtctcactttgttgcccaggctggtctcaaactcctggactcaagtgattctcccacctcagcctcccaaagtgctggggttacaggtgtgagccactgcacctggtcgatactgacttttttttttttttgagatggagttttgctctgttgcccaggctagagcgcagtggtgtgatctcagctcactgcaacctccacctcccaggttaaagggattcttctgcctcagtctcctgagtagctgggattacaggcaagtgccatcatgactggctaatttttgtatttttagcactatgtttagtactgtgttggccaggcttgtctcgaactcctgacctcaagtgatccacccacctcagcctcccaaagtgctgggattacaggtgtgagccaccgtaatcggccaacattgacatttttagtagactttttgtttgtttacttgcttattatctgctgccttccacactctggcgaaatcctgccacccacccacacacacataggcactgaatgggcagaactctgaaggccagaattttatatttcttttcactgtaaacatcatcatctgtcactgatggcacactaggatgctcagcaactgtgtgcatgaaggaagtaagcactagtttgtgaaggctgcaaaactcttgagtattctaagagttttggccaaaatgaatgtacagctttagtggcagaagctaatactcagaaattgaggccgtatattggataacacaggatttggatgattattttaaaataatattttacattgtatatatgtgtgtgtgtgtgtgtgtgtgtgtgtgtatgtgtgtgtgtgtgtatatatatatgtatgtatgtgtattagtccgttctcatgctgctatgaagaaatacctgagactgggtaatttataaaggaaagaggtttaattgactcacagttccacagagctggggaggcctcagaaaacttaacagttatggcagaaggggaagcaaacacatttttcttcacatggtggccggaattagaagaatgtgagccgagcaaaggggaaagccccttataaaaccatcagacatcgtgagaacttactattatgagaatagcgtgggggaaaccacccccacgattcaattacctcccaccaaatccctcccatgacatatgaggattatgggaactatgattcaagatgagatttgggtagggacacagccaaaccatatcagtatgtatatgtatacaagtattatatatatatgtatgtgtttgtatgcatacatgtattatatatggaggaaattctaattttgtaaaaaactggattgtgagttttaaggagatgttatataaagttaagacaatgtcattttgtggtattggtctgaattacaatgtagtttcttagtgatatttttcctttattcag

SEQ ID NO: 24 - DNA, 78 bp, Artificial Sequence
  Synthetic construct
cactccctctctgcgcgctcgctcgctcactgaggccgggcgaccaaaggtcgcccacgcccgggctttgcccgggcg

SEQ ID NO: 25 - DNA, 60 bp, Artificial Sequence
  Synthetic construct
tagcaagttaaaataaggctagtccgttatcaacttgaaaaagtggcaccgagtcggtgc

SEQ ID NO: 26 - protein, 7 aa, Simian vacuolating virus 40
PKKKRKV

SEQ ID NO: 27 - protein, 17 aa, Simian vacuolating virus 40
PKKKRKVEDPKKKRKVD

SEQ ID NO: 28 - DNA, 33 bp, Artificial Sequence
  Synthetic construct
gggaggattgggaagagaatagcaggcatgctg

SEQ ID NO: 29 - DNA, 33 bp, Artificial Sequence
  Synthetic construct
cagcatgcctgctattctcttcccaatcctccc

SEQ ID NO: 30 - DNA, 447 bp, Artificial Sequence
  Synthetic construct
cacatgtgagggcctatttcccatgattccttcatatttgcatatacgatacaaggctgttagagagataattggaattaatttgactgtaaacacaaagatattagtacaaaatacgtgacgtagaaagtaataatttcttgggtagtttgcagttttaaaattatgttttaaaatggactatcatatgcttaccgtaacttgaaagtatttcgatttcttggctttatatatcttgtggaaaggacgaaacaccgggtcttcgagaagacctgttttagagctagaaatagcaagttaaaataaggctagtccgttatcaacttgaaaaagtggcaccgagtcggtgcttttttgttttagagctagaaatagcaagttaaaataaggctagtccgtttttagcgcgtgcgccaattctgcagacaaatggctctagaggtaccc

SEQ ID NO: 31 - DNA, 20 bp, Artificial Sequence
  Synthetic construct
ttcatctgcactgccaagac

SEQ ID NO: 32 - DNA, 20 bp, Artificial Sequence
  Synthetic construct
tcgagttgtccacagtcagc

SEQ ID NO: 33 - DNA, 1153 bp, Artificial Sequence
  Synthetic construct
ctcacatgtgagggcctatttcccatgattccttcatatttgcatatacgatacaaggctgttagagagataattggaattaatttgactgtaaacacaaagatattagtacaaaatacgtgacgtagaaagtaataatttcttgggtagtttgcagttttaaaattatgttttaaaatggactatcatatgcttaccgtaacttgaaagtatttcgatttcttggctttatatatcttgtggaaaggacgaaacaccgggtcttcgagaagacctgttttagagctagaaatagcaagttaaaataaggctagtccgttatcaacttgaaaaagtggcaccgagtcggtgcttttttgttttagagctagaaatagcaagttaaaataaggctagtccgtttttagcgcgtgcgccaattctgcagacaaatggctctagagaccggcgccgctacaggctttccaccggtggtctcttctagaggtacccgttacatctagttattaatagtaatcaattacggggtcattagttcatagcccatatatggagttccgcgttacataacttacggtaaatggcccgcctggctgaccgcccaacgacccccgcccattgacgtcaataatgacgtatgttcccatagtaacgccaatagggactttccattgacgtcaatgggtggagtatttacggtaaactgcccacttggcagtacatcaagtgtatcatatgccaagtacgccccctattgacgtcaatgacggtaaatggcccgcctggcattatgcccagtacatgaccttatgggactttcctacttggcagtacatctacgtattagtcatcgctattaccatggtgatgcggttttggcagtacatcaatgggcgtggatagcggtttgactcacggggatttccaagtctccaccccattgacgtcaatgggagtttgttttggcaccaaaatcaacgggactttccaaaatgtcgtaacaactccgccccattgacgcaaatgggcggtaggcgtgtacggtgggaggtctatataagcagagctctctggctaactagagaacccactgcttactggcttatcgaaattaatacgactcactatagggagaaccaagctggctagccgc

SEQ ID NO: 34 - DNA, 45 bp, Artificial Sequence
  Synthetic construct
ataacatgtggtctcactctagaggcatgtgagggcctatttccc

SEQ ID NO: 35 - DNA, 36 bp, Artificial Sequence
  Synthetic construct
tatggtaccggtctcatagagccatttgtctgcaga

SEQ ID NO: 36 - DNA, 24 bp, Artificial Sequence
  Synthetic construct
caccgcactaccagagctaactca

SEQ ID NO: 37 - DNA, 24 bp, Artificial Sequence
  Synthetic construct
aaactgagttagctctggtagtgc

SEQ ID NO: 38 - DNA, 24 bp, Artificial Sequence
  Synthetic construct
caccgtgcgaatacgccacgcgat

SEQ ID NO: 39 - DNA, 24 bp, Artificial Sequence
  Synthetic construct
aaacatcgcgtggcgtattcgcac

SEQ ID NO: 40 - protein, 1368 aa, Streptococcus pyogenes [sequence omitted]

SEQ ID NO: 41 - DNA, 20 bp, Artificial Sequence
  Synthetic construct
ggcgggtggatcacgagttc

SEQ ID NO: 42 - DNA, 20 bp, Artificial Sequence
  Synthetic construct
aaagctaccggttacctgaa

SEQ ID NO: 43 - DNA, 20 bp, Artificial Sequence
  Synthetic construct
tcattcttgtggcagtaagg

SEQ ID NO: 44 - DNA, 20 bp, Artificial Sequence
  Synthetic construct
ggagtcacatgggagtcaca

SEQ ID NO: 45 - DNA, 21 bp, Artificial Sequence
  Synthetic construct
tttaacgttatcattttccca

SEQ ID NO: 46 - DNA, 21 bp, Artificial Sequence
  Synthetic construct
agtttcattctgtcacccagg

SEQ ID NO: 47 - DNA, 21 bp, Artificial Sequence
  Synthetic construct
aaaaattagccgggcatgatg

SEQ ID NO: 48 - DNA, 21 bp, Artificial Sequence
  Synthetic construct
tgtaagactggagatagagac

SEQ ID NO: 49 - DNA, 21 bp, Artificial Sequence
  Synthetic construct
cttttgacagtttttaaggcg

SEQ ID NO: 50 - DNA, 103 bp, Artificial Sequence
  Synthetic construct
gtttaacgttatcattttcccagttttagtactctggaaacagaatctactaaaacaaggcaaaatgccgtgtttatctcgtcaacttgttggcgagattttt

SEQ ID NO: 51 - DNA, 103 bp, Artificial Sequence
  Synthetic construct
gagtttcattctgtcacccagggttttagtactctggaaacagaatctactaaaacaaggcaaaatgccgtgtttatctcgtcaacttgttggcgagattttt

SEQ ID NO: 52 - DNA, 103 bp, Artificial Sequence
  Synthetic construct
gaaaaattagccgggcatgatggttttagtactctggaaacagaatctactaaaacaaggcaaaatgccgtgtttatctcgtcaacttgttggcgagattttt

SEQ ID NO: 53 - DNA, 103 bp, Artificial Sequence
  Synthetic construct
gtgtaagactggagatagagacgttttagtactctggaaacagaatctactaaaacaaggcaaaatgccgtgtttatctcgtcaacttgttggcgagattttt

SEQ ID NO: 54 - DNA, 103 bp, Artificial Sequence
  Synthetic construct
gcttttgacagtttttaaggcggttttagtactctggaaacagaatctactaaaacaaggcaaaatgccgtgtttatctcgtcaacttgttggcgagattttt

SEQ ID NO: 55 - protein, 1053 aa, Staphylococcus aureus
MKRNYILGLDIGITSVGYGIIDYETRDVIDAGVRLFKEANVENNEGRRSKRGARRLKRRRRHRIQRVKKLLFDYNLLTDHSELSGINPYEARVKGLSQKLSEEEFSAALLHLAKRRGVHNVNEVEEDTGNELSTKEQISRNSKALEEKYVAELQLERLKKDGEVRGSINRFKTSDYVKEAKQLLKVQKAYHQLDQSFIDTYIDLLETRRTYYEGPGEGSPFGWKDIKEWYEMLMGHCTYFPEELRSVKYAYNADLYNALNDLNNLVITRDENEKLEYYEKFQIIENVFKQKKKPTLKQIAKEILVNEEDIKGYRVTSTGKPEFTNLKVYHDIKDITARKEIIENAELLDQIAKILTIYQSSEDIQEELTNLNSELTQEEIEQISNLKGYTGTHNLSLKAINLILDELWHTNDNQIAIFNRLKLVPKKVDLSQQKEIPTTLVDDFILSPVVKRSFIQSIKVINAIIKKYGLPNDIIIELAREKNSKDAQKMINEMQKRNRQTNERIEEIIRTTGKENAKYLIEKIKLHDMQEGKCLYSLEAIPLEDLLNNPFNYEVDHIIPRSVSFDNSFNNKVLVKQEENSKKGNRTPFQYLSSSDSKISYETFKKHILNLAKGKGRISKTKKEYLLEERDINRFSVQKDFINRNLVDTRYATRGLMNLLRSYFRVNNLDVKVKSINGGFTSFLRRKWKFKKERNKGYKHHAEDALIIANADFIFKEWKKLDKAKKVMENQMFEEKQAESMPEIETEQEYKEIFITPHQIKHIKDFKDYKYSHRVDKKPNRELINDTLYSTRKDDKGNTLIVNNLNGLYDKDNDKLKKLINKSPEKLLMYHHDPQTYQKLKLIMEQYGDEKNPLYKYYEETGNYLTKYSKKDNGPVIKKIKYYGNKLNAHLDITDDYPNSRNKVVKLSLKPYRFDVYLDNGVYKFVTVKNLDVIKKENYYEVNSKCYEEAKKLKKISNQAEFIASFYNNDLIKINGELYRVIGVNNDLLNRIEVNMIDITYREYLENMNDKRPPRIIKTIASKTQSIKKYSTDILGNLYEVKSKKHPQIIKKG

SEQ ID NO: 56 - DNA, 321 bp, Artificial Sequence
  Synthetic construct
tatacgcgtgttgacactagttcgcgaaatattgactcacggggatttccaagtctccaccccattgacgtcaatgggagtttgttttggcaccaaaatcaacgggactttccaaaatgtcgtaacaactccgccccattgacgcaaatgggcggtaggcgtgtacggtgggaggtctatataagcagagctcgtttagtgaaccgtcagatcgccgccaccatggacaagaagtacagcatcggcctggacatcggcaccaactctgtgggctgggccgtgatcaccgacgagtacaaggtgcccagcaagaaattcaag

SEQ ID NO: 57 - DNA, 168 bp, Artificial Sequence
  Synthetic construct
tgactcgagaacttgtttattgcagcttataatggttacaaataaagcaatagcatcacaaatttcacaaataaagcatttttttcactgcattctagttgtggtttgtccaaactcatcaatgtatcttatcatgtctgcaatatttcgcgagaagacaatagcagg

SEQ ID NO: 58 - DNA, 23 bp, Artificial Sequence
  Synthetic construct
ggcgggtggatcacgagttcagg

SEQ ID NO: 59 - DNA, 23 bp, Artificial Sequence
  Synthetic construct
ggagtcacatgggagtcacaggg

SEQ ID NO: 60 - DNA, 324 bp, Artificial Sequence
  Synthetic construct
ctagtggcggccgctcgagcatgcatctagagggccctattctatagtgtcacctaaatgctagagctcgctgatcagcctcgactgtgccttctagttgccagccatctgttgtttgcccctcccccgtgccttccttgaccctggaaggtgccactcccactgtcctttcctaataaaatgaggaaattgcatcgcattgtctgagtaggtgtcattctattctggggggtggggtggggcaggacagcaagggggaggattgggaagacaatagcaggcatgctggggagctagagtcgaccggaccgctgcaggcatgca

SEQ ID NO: 61 - DNA, 20 bp, Artificial Sequence
  Synthetic construct
gcataaggactaaagaccta

SEQ ID NO: 62 - DNA, 20 bp, Artificial Sequence
  Synthetic construct
ggtagtggttgaactcacaa

SEQ ID NO: 63 - DNA, 2471 bp, Artificial Sequence
  Synthetic construct
gggccccagaagcctggtggttgtttgtccttctcaggggaaaagtgaggcggccccttggaggaaggggccgggcagaatgatctaatcggattccaagcagctcaggggattgtctttttctagcaccttcttgccactcctaagcgtcctccgtgaccccggctgggatttagcctggtgctgtgtcagccccggtctcccaggggcttcccagtggtccccaggaaccctcgacagggcccggtctctctcgtccagcaagggcagggacgggccacaggccaagggcggagtcgctgcgacgctgccttcgccccgtgccccgctccgccgccgcctcgcgccgcccgccccggctctgactgaccgcgttactcccacaggtgagcgggcgggacggcccttctcctccgggctgtaattagcgcttggtttaatgacggcttgtttcttttctgtggctgcgtgaaagccttgaggggctccgggagggccctttgtgcggggggagcggctcggggggtgcgtgcgtgtgtgtgtgcgtggggagcgccgcgtgcggctccgcgctgcccggcggctgtgagcgctgcgggcgcggcgcggggctttgtgcgctccgcagtgtgcgcgaggggagcgcggccgggggcggtgccccgcggtgcggggggggctgcgaggggaacaaaggctgcgtgcggggtgtgtgcgtgggggggtgagcagggggtgtgggcgcgtcggtcgggctgcaaccccccctgcacccccctccccgagttgctgagcacggcccggcttcgggtgcggggctccgtacggggcgtggcgcggggctcgccgtgccgggcggggggtggcggcaggtgggggtgccgggcggggcggggccgcctcgggccggggagggctcgggggaggggcgcggcggcccccggagcgccggcggctgtcgaggcgcggcgagccgcagccattgccttttatggtaatcgtgcgagagggcgcagggacttcctttgtcccaaatctgtgcggagccgaaatctgggaggcgccgccgcaccccctctagcgggcgcggggcgaagcggtgcggcgccggcaggaaggaaatgggcggggagggccttcgtgcgtcgccgcgccgccgtccccttctccctctccagcctcggggctgtccgcggggggacggctgccttcgggggggacggggcagggcggggttcggcttctggcgtgtgaccggcggctctagagcctctgctaaccatgttcatgccttcttctttttcctacagctcctgggcaacgtgctggttattgtgctgtctcatcattttggcaaagaattcttcgaaagatctgctagcttaattaacccggtcgccaccatggtgagcaagggcgaggagctgttcaccggggtggtgcccatcctggtcgagctggacggcgacgtaaacggccacaagttcagcgtgtccggcgagggcgagggcgatgccacctacggcaagctgaccctgaagttcatctgcaccaccggcaagctgcccgtgccctggcccaccctcgtgaccaccctgacctacggcgtgcagtgcttcagccgctaccccgaccacatgaagcagcacgacttcttcaagtccgccatgcccgaaggctacgtccaggagcgcaccatcttcttcaaggacgacggcaactacaagacccgcgccgaggtgaagttcgagggcgacaccctggtgaaccgcatcgagctgaagggcatcgacttcaaggaggacggcaacatcctggggcacaagctggagtacaactacaacagccacaacgtctatatcatggccgacaagcagaagaacggcatcaaggtgaacttcaagatccgccacaacatcgaggacggcagcgtgcagctcgccgaccactaccagcagaacacccccatcggcgacggccccgtgctgctgcccgacaaccactacctgagcacccagtccgccctgagcaaagaccccaacgagaagcgcgatcacatggtcctgctggagttcgtgaccgccgccgggatcactctcggcatggacgagctgtacaagtaaagcggccaaatcgtacgcctaggtgatcaagatctgctagcttaattaacccgggactagtggcggccgctcgagcatgcatctagagggccctattctatagtgtcacctaaatgctagagctcgctgatcagcctcgactgtgccttctagttgccagccatctgttgtttgcccctcccccgtgccttccttgaccctggaaggtgccactcccactgtcctttcctaataaaatgaggaaattgcatcgcattgtctgagtaggtgtcattctattctggggggtggggtggggcaggacagcaagggggaggattgggaagacaatagcaggcatgctgggga

SEQ ID NO: 64 - DNA, 20 bp, Artificial Sequence
  Synthetic construct
cccctcgcctgtactgaaag

SEQ ID NO: 65 - DNA, 20 bp, Artificial Sequence
  Synthetic construct
gcacatcatctgaggcaggt

SEQ ID NO: 66 - DNA, 4009 bp, Artificial Sequence
  Synthetic construct
atgaattctctagacaattggactcacggggatttccaagtctccaccccattgacgtcaatgggagtttgttttggcaccaaaatcaacgggactttccaaaatgtcgtaacaactccgccccattgacgcaaatgggcggtaggcgtgtacggtgggaggtctatataagcagagctcgtttagtgaaccgtcagatcacgcgtgccaccatgaagcggaactacatcctgggcctggacatcggcatcaccagcgtgggctacggcatcatcgactacgagacacgggacgtgatcgatgccggcgtgcggctgttcaaagaggccaacgtggaaaacaacgagggcaggcggagcaagagaggcgccagaaggctgaagcggcggaggcggcatagaatccagagagtgaagaagctgctgttcgactacaacctgctgaccgaccacagcgagctgagcggcatcaacccctacgaggccagagtgaagggcctgagccagaagctgagcgaggaagagttctctgccgccctgctgcacctggccaagagaagaggcgtgcacaacgtgaacgaggtggaagaggacaccggcaacgagctgtccaccaaagagcagatcagccggaacagcaaggccctggaagagaaatacgtggccgaactgcagctggaacggctgaagaaagacggcgaagtgcggggcagcatcaacagattcaagaccagcgactacgtgaaagaagccaaacagctgctgaaggtgcagaaggcctaccaccagctggaccagagcttcatcgacacctacatcgacctgctggaaacccggcggacctactatgagggacctggcgagggcagccccttcggctggaaggacatcaaagaatggtacgagatgctgatgggccactgcacctacttccccgaggaactgcggagcgtgaagtacgcctacaacgccgacctgtacaacgccctgaacgacctgaacaatctcgtgatcaccagggacgagaacgagaagctggaatattacgagaagttccagatcatcgagaacgtgttcaagcagaagaagaagcccaccctgaagcagatcgccaaagaaatcctcgtgaacgaagaggatattaagggctacagagtgaccagcaccggcaagcccgagttcaccaacctgaaggtgtaccacgacatcaaggacattaccgcccggaaagagattattgagaacgccgagctgctggatcagattgccaagatcctgaccatctaccagagcagcgaggacatccaggaagaactgaccaatctgaactccgagctgacccaggaagagatcgagcagatctctaatctgaagggctataccggcacccacaacctgagcctgaaggccatcaacctgatcctggacgagctgtggcacaccaacgacaaccagatcgctatcttcaaccggctgaagctggtgcccaagaaggtggacctgtcccagcagaaagagatccccaccaccctggtggacgacttcatcctgagccccgtcgtgaagagaagcttcatccagagcatcaaagtgatcaacgccatcatcaagaagtacggcctgcccaacgacatcattatcgagctggcccgcgagaagaactccaaggacgcccagaaaatgatcaacgagatgcagaagcggaaccggcagaccaacgagcggatcgaggaaatcatccggaccaccggcaaagagaacgccaagtacctgatcgagaagatcaagctgcacgacatgcaggaaggcaagtgcctgtacagcctggaagccatccctctggaagatctgctgaacaaccccttcaactatgaggtggaccacatcatccccagaagcgtgtccttcgacaacagcttcaacaacaaggtgctcgtgaagcaggaagaaaacagcaagaagggcaaccggaccccattccagtacctgagcagcagcgacagcaagatcagctacgaaaccttcaagaagcacatcctgaatctggccaagggcaagggcagaatcagcaagaccaagaaagagtatctgctggaagaacgggacatcaacaggttctccgtgcagaaagacttcatcaaccggaacctggtggataccagatacgccaccagaggcctgatgaacctgctgcggagctacttcagagtgaacaacctggacgtgaaagtgaagtccatcaatggcggcttcaccagctttctgcggcggaagtggaagtttaagaaagagcggaacaaggggtacaagcaccacgccgaggacgccctgatcattgccaacgccgatttcatcttcaaagagtggaagaaactggacaaggccaaaaaagtgatggaaaaccagatgttcgaggaaaagcaggccgagagcatgcccgagatcgaaaccgagcaggagtacaaagagatcttcatcaccccccaccagatcaagcacattaaggacttcaaggactacaagtacagccaccgggtggacaagaagcctaatagagagctgattaacgacaccctgtactccacccggaaggacgacaagggcaacaccctgatcgtgaacaatctgaacggcctgtacgacaaggacaatgacaagctgaaaaagctgatcaacaagagccccgaaaagctgctgatgtaccaccacgacccccagacctaccagaaactgaagctgattatggaacagtacggcgacgagaagaatcccctgtacaagtactacgaggaaaccgggaactacctgaccaagtactccaaaaaggacaacggccccgtgatcaagaagattaagtattacggcaacaaactgaacgcccatctggacatcaccgacgactaccccaacagcagaaacaaggtcgtgaagctgtccctgaagccctacagattcgacgtgtacctggacaatggcgtgtacaagttcgtgaccgtgaagaatctggatgtgatcaaaaaagaaaactactacgaagtgaatagcaagtgctatgaggaagctaagaagctgaagaagatcagcaaccaggccgagtttatcgcctccttctacaacaacgatctgatcaagatcaacggcgagctgtatagagtgatcggcgtgaacaacgacctgctgaaccggatcgaagtgaacatgatcgacatcacctaccgcgagtacctggaaaacatgaacgacaagaggccccccaggatcattaagacaatcgcctccaagacccagagcattaagaagtacagcacagacattctgggcaacctgtatgaagtgaaatctaagaagcaccctcagatcatcaaaaagggcggatcccccaagaaaaagcgcaaagtggactacaaagacgatgacgacaagtgagctagcgactgtgccttctagttgccagccatctgttgtttgcccctcccccgtgccttccttgaccctggaaggtgccactcccactgtcctttcctaataaaatgaggaaattgcatcgcattgtctgagtaggtgtcattctattctggggggtggggtggggcaggacagcaagggggaggattgggaagagaatagcaggcatgctggtacctgagggcctatttcccatgattccttcatatttgcatatacgatacaaggctgttagagagataattggaattaatttgactgtaaacacaaagatattagtacaaaatacgtgacgtagaaagtaataatttcttgggtagtttgcagttttaaaattatgttttaaaatggactatcatatgcttaccgtaacttgaaagtatttcgatttcttggctttatatatcttgtggaaaggacgaaacaccggagaccacggcaggtctcagttttagtactctggaaacagaatctactaaaacaaggcaaaatgccgtgtttatctcgtcaacttgttggcgagatttttgcggccgcgtcgacat